European Patent Application EP 4 810 151 A1, published September 23, 2026. Title: 생물학적 고분자 합성을 위한 복합 고체 지지체. Applicant: 에스피투티엑스주식회사. The sequence listing filed with the application follows.

SEQUENCE LISTING (3 sequences)

SEQ ID NO: 1 - protein, 10 aa, unidentified
VQAAIDYING

SEQ ID NO: 2 - protein, 10 aa, unidentified
WFTTLISTIM

SEQ ID NO: 3 - skipped